European Patent Specification EP 3 164 415 B1, published October 30, 2024. Title: ANTI- MGLUR2 CONFORMATIONAL SINGLE DOMAIN ANTIBODIES AND USES THEREOF. Applicant: INSERM. The sequence listing filed with the application follows.

SEQUENCE LISTING (18 sequences)

SEQ ID NO: 1 - protein, 8 aa, Artificial
  DN7 CDR1
GRTFRPYG

SEQ ID NO: 2 - protein, 8 aa, Artificial
  DN7 CDR2
IIWSLGYT

SEQ ID NO: 3 - protein, 12 aa, Artificial
  DN7 CDR3
AARDRSSSEYDY

SEQ ID NO: 4 - protein, 119 aa, Artificial
  DN7 single domain antibody
QVQLVQSGGGYVQAGGSLSVSCAASGRTFRPYGVGWFRQAPGKEREFVAAIIWSLGYTIYADSVKGRFTISRDNAKNTVYLQMNSLKAEDTAVYYCAARDRSSSEYDYWGQGTQVTVSS

SEQ ID NO: 5 - protein, 8 aa, Artificial
  DN10 CDR1
GRTDSIYS

SEQ ID NO: 6 - protein, 7 aa, Artificial
  DN10 CDR2
ITWREYT

SEQ ID NO: 7 - protein, 12 aa, Artificial
  DN10 CDR3
ALRPGLRDDLNY

SEQ ID NO: 8 - protein, 119 aa, Artificial
  DN10 single domain antibody
EVQLVESGGGVVQPGDSLRLSCVASGRTDSIYSMAWFRQAPGKEREFVAIITWRREYTNYEDSVRGRFTISRDNAKNAVYLQMNKLKPEDTAVYYCALRPGLRDDLNYWGQGTQVTVSS

SEQ ID NO: 9 - protein, 8 aa, Artificial
  DN13 CDR1
VRFFSINT

SEQ ID NO: 10 - protein, 7 aa, Artificial
  DN13 CDR2
ITSSGST

SEQ ID NO: 11 - protein, 12 aa, Artificial
  DN13 CDR3
HADYKYTTHNTA

SEQ ID NO: 12 - protein, 118 aa, Artificial
  DN13 single domain antibody
QVQLVQSGGGLVQAGGSLRLSCAASVRFFSINTMGWYRQAPGKQRELVADITSSGSTNYADSGKGRFTISRDNAKNTVYLQMNRLKPEDTAVYYCHADYKYTTHNTAWGQGTQVTVSS

SEQ ID NO: 13 - protein, 15 aa, Artificial
  linker
GGGGSGGGGSGGGGS

SEQ ID NO: 14 - protein, 20 aa, Artificial
  linker
GGGGSGGGGSGGGGSGGGGS

SEQ ID NO: 15 - protein, 5 aa, Artificial
  linker
GGGGS

SEQ ID NO: 16 - protein, 3 aa, Artificial
  linker
GGS

SEQ ID NO: 17 - protein, 3 aa, Artificial
  linker
GGG

SEQ ID NO: 18 - protein, 15 aa, Artificial
  linker
GGGSSGGGSSGGGSS